European Patent Specification EP 3 941 206 B1, published September 30, 2026. Title: NOUVELLES UTILISATIONS D'UNE LACTONASE MUTEE ET COMPOSITIONS. Applicant: Fondation Méditerranée Infection Aix-Marseille Université Gene & Green TK. The sequence listing filed with the application follows.

SEQUENCE LISTING (30 sequences)

SEQ ID NO: 1 - protein, 314 aa, Sulfolobus solfataricus
MRIPLVGKDSIESKDIGFTLIHEHLRVFSEAVRQQWPHLYNEDEEFRNAVNEVKRAMQFGVKTIVDPTVMGLGRDIRFMEKVVKATGINLVAGTGIYIYIDLPFYFLNRSIDEIADLFIHDIKEGIQGTLNKAGFVKIAADEPGITKDVEKVIRAAAIANKETKVPIITHSNAHNNTGLEQQRILTEEGVDPGKILIGHLGDTDNIDYIKKIADKGSFIGLDRYGLDLFLPVDKRNETTLRLIKDGYSDKIMISHDYCCTIDWGTAKPEYKPKLAPRWSITLIFEDTIPFLKRNGVNEEVIATIFKENPKKFFS

SEQ ID NO: 2 - protein, 314 aa, Sulfolobus solfataricus
MRIPLVGKDSIESKDIGFTLIHEHLRVFSEAVRQQWPHLYNEDEEFRNAVNEVKRAMQFGVKTIVDPTVMGLGRDIRFMEKVVKATGINLVAGTGIYIYIDLPFYFLNRSIDEIADLFIHDIKEGIQGTLNKAGFVKIAADEPGITKDVEKVIRAAAIANKETKVPIITHSNAHNNTGLEQQRILTEEGVDPGKILIGHLGDTDNIDYIKKIADKGSFIGLDRYGLDLFLPVDKRNETTLRLIKDGYSDKIMISHDYCCTIDIGTAKPEYKPKLAPRWSITLIFEDTIPFLKRNGVNEEVIATIFKENPKKFFS

SEQ ID NO: 3 - DNA, 20 bp, Artificial sequence
  amorce
tcaaggactcgctgatcctg

SEQ ID NO: 4 - DNA, 20 bp, Artificial sequence
  amorce
gatcatgaagtccagggcct

SEQ ID NO: 5 - DNA, 20 bp, Artificial sequence
  amorce
ggttgatcgtcagccatcat

SEQ ID NO: 6 - DNA, 19 bp, Artificial sequence
  amorce
ggccttttcttttgcgtct

SEQ ID NO: 7 - DNA, 20 bp, Artificial sequence
  amorce
tcttcgagcatgacttcgga

SEQ ID NO: 8 - DNA, 20 bp, Artificial sequence
  amorce
tggcgaggttgttatggact

SEQ ID NO: 9 - DNA, 20 bp, Artificial sequence
  amorce
cgtccgaagaagaagcatcg

SEQ ID NO: 10 - DNA, 20 bp, Artificial sequence
  amorce
cgcagcggtgtttctctatc

SEQ ID NO: 11 - DNA, 19 bp, Artificial sequence
  amorce
aagaccaaggaccgtgacc

SEQ ID NO: 12 - DNA, 20 bp, Artificial sequence
  amorce
agccctgatcgttcacgtag

SEQ ID NO: 13 - DNA, 19 bp, Artificial sequence
  amorce
acaggatcggcgtgagctt

SEQ ID NO: 14 - DNA, 18 bp, Artificial sequence
  amorce
ccgcaacccttccagcca

SEQ ID NO: 15 - DNA, 20 bp, Artificial sequence
  amorce
gaaccacctgatcccttccc

SEQ ID NO: 16 - DNA, 20 bp, Artificial sequence
  amorce
taggagcttgacgatgacct

SEQ ID NO: 17 - DNA, 19 bp, Artificial sequence
  amorce
caggatggctgcgtctttg

SEQ ID NO: 18 - DNA, 18 bp, Artificial sequence
  amorce
aactacctggcctacggc

SEQ ID NO: 19 - DNA, 18 bp, Artificial sequence
  amorce
ggacaggtaggaggcttg

SEQ ID NO: 20 - DNA, 18 bp, Artificial sequence
  amorce
tacgcgagcaagtgaccc

SEQ ID NO: 21 - DNA, 18 bp, Artificial sequence
  amorce
ggaattccgcctccgcca

SEQ ID NO: 22 - DNA, 18 bp, Artificial sequence
  amorce
gccgacagcgatgaagac

SEQ ID NO: 23 - DNA, 19 bp, Artificial sequence
  amorce
tcaccggcctgatgacggc

SEQ ID NO: 24 - DNA, 19 bp, Artificial sequence
  amorce
gaagcgctggatgtagtcg

SEQ ID NO: 25 - DNA, 19 bp, Artificial sequence
  amorce
gcgagtacaggctttccac

SEQ ID NO: 26 - DNA, 19 bp, Artificial sequence
  amorce
aaaccatctggcggcactc

SEQ ID NO: 27 - DNA, 18 bp, Artificial sequence
  amorce
cggaagcattggccggtg

SEQ ID NO: 28 - DNA, 17 bp, Artificial sequence
  amorce
cgcgcgacaggctgatg

SEQ ID NO: 29 - DNA, 18 bp, Artificial sequence
  amorce
ctggtggccatagcgagg

SEQ ID NO: 30 - DNA, 19 bp, Artificial sequence
  amorce
gtctggcggtgtcctactt